European Patent Specification EP 3 472 338 B1, published May 22, 2024. Title: Means and methods for modifying multiple alleles. Applicant: Glycotope GmbH. The sequence listing filed with the application follows.

SEQUENCE LISTING (16 sequences)

SEQ ID NO: 1 - DNA, 19 bp, artificial
  targeting sequence for B4GALNT3
attgctgcagatgacaacg

SEQ ID NO: 2 - DNA, 19 bp, artificial
  targeting sequence for B4GALNT3
tggattttccctgggcagc

SEQ ID NO: 3 - DNA, 19 bp, artificial
  targeting sequence for B4GALNT3
cccgggacaccctctatcg

SEQ ID NO: 4 - DNA, 20 bp, artificial
  targeting sequence for B4GALNT3
ggccgaagcatgtcagcggg

SEQ ID NO: 5 - DNA, 19 bp, artificial
  targeting sequence for B4GALNT4
gcgtgcacttgtgtattcg

SEQ ID NO: 6 - DNA, 19 bp, artificial
  targeting sequence for B4GALNT4
ccacagtcactcaccgcct

SEQ ID NO: 7 - DNA, 19 bp, artificial
  targeting sequence for B4GALNT4
ggtttcatccacccggcga

SEQ ID NO: 8 - DNA, 20 bp, artificial
  targeting sequence for B4GALNT4
gagtccatagttcttccact

SEQ ID NO: 9 - DNA, 351 bp, artificial
  B4GALNT3 gRNA plasmid Exon6 1(+)
gagggcctatttcccatgattccttcatatttgcatatacgatacaaggctgttagagagataattggaattaatttgactgtaaacacaaagatattagtacaaaatacgtgacgtagaaagtaataatttcttgggtagtttgcagttttaaaattatgttttaaaatggactatcatatgcttaccgtaacttgaaagtatttcgatttcttggctttatatatcttgtggaaaggacgaaacaccgattgctgcagatgacaacggttttagagctagaaatagcaagttaaaataaggctagtccgttatcaacttgaaaaagtggcaccgagtcggtgctttttt

SEQ ID NO: 10 - DNA, 351 bp, artificial
  B4GALNT3 gRNA plasmid Exon6 1(-)
gagggcctatttcccatgattccttcatatttgcatatacgatacaaggctgttagagagataattggaattaatttgactgtaaacacaaagatattagtacaaaatacgtgacgtagaaagtaataatttcttgggtagtttgcagttttaaaattatgttttaaaatggactatcatatgcttaccgtaacttgaaagtatttcgatttcttggctttatatatcttgtggaaaggacgaaacaccgtggattttccctgggcagcgttttagagctagaaatagcaagttaaaataaggctagtccgttatcaacttgaaaaagtggcaccgagtcggtgctttttt

SEQ ID NO: 11 - DNA, 351 bp, artificial
  B4GALNT3 gRNA plasmid Exon10 2(+)
gagggcctatttcccatgattccttcatatttgcatatacgatacaaggctgttagagagataattggaattaatttgactgtaaacacaaagatattagtacaaaatacgtgacgtagaaagtaataatttcttgggtagtttgcagttttaaaattatgttttaaaatggactatcatatgcttaccgtaacttgaaagtatttcgatttcttggctttatatatcttgtggaaaggacgaaacaccgcccgggacaccctctatcggttttagagctagaaatagcaagttaaaataaggctagtccgttatcaacttgaaaaagtggcaccgagtcggtgctttttt

SEQ ID NO: 12 - DNA, 351 bp, artificial
  B4GALNT3 gRNA plasmid Exon10 2(-)
gagggcctatttcccatgattccttcatatttgcatatacgatacaaggctgttagagagataattggaattaatttgactgtaaacacaaagatattagtacaaaatacgtgacgtagaaagtaataatttcttgggtagtttgcagttttaaaattatgttttaaaatggactatcatatgcttaccgtaacttgaaagtatttcgatttcttggctttatatatcttgtggaaaggacgaaacaccggccgaagcatgtcagcggggttttagagctagaaatagcaagttaaaataaggctagtccgttatcaacttgaaaaagtggcaccgagtcggtgctttttt

SEQ ID NO: 13 - DNA, 351 bp, artificial
  B4GALNT4 gRNA plasmid Exon7 1(+)
gagggcctatttcccatgattccttcatatttgcatatacgatacaaggctgttagagagataattggaattaatttgactgtaaacacaaagatattagtacaaaatacgtgacgtagaaagtaataatttcttgggtagtttgcagttttaaaattatgttttaaaatggactatcatatgcttaccgtaacttgaaagtatttcgatttcttggctttatatatcttgtggaaaggacgaaacaccggcgtgcacttgtgtattcggttttagagctagaaatagcaagttaaaataaggctagtccgttatcaacttgaaaaagtggcaccgagtcggtgctttttt

SEQ ID NO: 14 - DNA, 351 bp, artificial
  B4GALNT4 gRNA plasmid Exon7 1(-)
gagggcctatttcccatgattccttcatatttgcatatacgatacaaggctgttagagagataattggaattaatttgactgtaaacacaaagatattagtacaaaatacgtgacgtagaaagtaataatttcttgggtagtttgcagttttaaaattatgttttaaaatggactatcatatgcttaccgtaacttgaaagtatttcgatttcttggctttatatatcttgtggaaaggacgaaacaccgccacagtcactcaccgcctgttttagagctagaaatagcaagttaaaataaggctagtccgttatcaacttgaaaaagtggcaccgagtcggtgctttttt

SEQ ID NO: 15 - DNA, 351 bp, artificial
  B4GALNT4 gRNA plasmid Exon4-6 2(+)
gagggcctatttcccatgattccttcatatttgcatatacgatacaaggctgttagagagataattggaattaatttgactgtaaacacaaagatattagtacaaaatacgtgacgtagaaagtaataatttcttgggtagtttgcagttttaaaattatgttttaaaatggactatcatatgcttaccgtaacttgaaagtatttcgatttcttggctttatatatcttgtggaaaggacgaaacaccgggtttcatccacccggcgagttttagagctagaaatagcaagttaaaataaggctagtccgttatcaacttgaaaaagtggcaccgagtcggtgctttttt

SEQ ID NO: 16 - DNA, 351 bp, artificial
  B4GALNT4 gRNA plasmid Exon4-6 2(-)
gagggcctatttcccatgattccttcatatttgcatatacgatacaaggctgttagagagataattggaattaatttgactgtaaacacaaagatattagtacaaaatacgtgacgtagaaagtaataatttcttgggtagtttgcagttttaaaattatgttttaaaatggactatcatatgcttaccgtaacttgaaagtatttcgatttcttggctttatatatcttgtggaaaggacgaaacaccgagtccatagttcttccactgttttagagctagaaatagcaagttaaaataaggctagtccgttatcaacttgaaaaagtggcaccgagtcggtgctttttt